European Patent Application EP 4 763 996 A1, published June 24, 2026. Title: 유전자의 복제수 및 유전자 변이형의 동시 결정 방법 및 킷트. Applicant: GENOTECH CORP. Application WO. The sequence listing filed with the application follows.

SEQUENCE LISTING (29 sequences)

SEQ ID NO: 1 - DNA, 25 bp, synthetic construct
  source 1..25: mol_type = other DNA
ggtaccgctggcactttctgttatg

SEQ ID NO: 2 - DNA, 24 bp, synthetic construct
  source 1..24: mol_type = other DNA
actagtgggagaagaaggaaggga

SEQ ID NO: 3 - DNA, 18 bp, synthetic construct
  source 1..18: mol_type = other DNA
ccacagccctgcggcacc

SEQ ID NO: 4 - DNA, 18 bp, synthetic construct
  source 1..18: mol_type = other DNA
tggtcaaccccctgccac

SEQ ID NO: 5 - DNA, 23 bp, synthetic construct
  source 1..23: mol_type = other DNA
tcaccctaataaaacccagacct

SEQ ID NO: 6 - DNA, 19 bp, synthetic construct
  source 1..19: mol_type = other DNA
ggacccggatgctgaaact

SEQ ID NO: 7 - DNA, 21 bp, synthetic construct
  source 1..21: mol_type = other DNA
acagtcaacacagcaggttca

SEQ ID NO: 8 - DNA, 20 bp, synthetic construct
  source 1..20: mol_type = other DNA
ctgtttcatgtccacgaccc

SEQ ID NO: 9 - DNA, 27 bp, synthetic construct
  misc_difference order(5,16)
  source 1..27: mol_type = other DNA
  modified_base order(5,16): mod_base = i; mod_base = i
aggtnattatgtaatnagccaaagtcc

SEQ ID NO: 10 - DNA, 22 bp, synthetic construct
  source 1..22: mol_type = other DNA
  misc_difference 13
  modified_base 13: mod_base = i; mod_base = i
acagtcaggcagnccagcaagg

SEQ ID NO: 11 - DNA, 23 bp, synthetic construct
  source 1..23: mol_type = other DNA
ctgaggccagcatggtggtagtg

SEQ ID NO: 12 - DNA, 28 bp, synthetic construct
  source 1..28: mol_type = other DNA
ggaggtgaaatgaggtaattatgtagtc

SEQ ID NO: 13 - DNA, 22 bp, synthetic construct
  source 1..22: mol_type = other DNA
ttcaggcagtataaaggcaaac

SEQ ID NO: 14 - DNA, 22 bp, synthetic construct
  source 1..22: mol_type = other DNA
ttcaggcagtagaaaggcaaac

SEQ ID NO: 15 - DNA, 22 bp, synthetic construct
  source 1..22: mol_type = other DNA
ttcaggcagtataaaggcaaac

SEQ ID NO: 16 - DNA, 24 bp, synthetic construct
  source 1..24: mol_type = other DNA
cctgaggccagcatggtggtagtg

SEQ ID NO: 17 - DNA, 20 bp, synthetic construct
  source 1..20: mol_type = other DNA
aggcttgctgtttgggctct

SEQ ID NO: 18 - DNA, 25 bp, synthetic construct
  source 1..25: mol_type = other DNA
tgacttgcttttaacatgaccattc

SEQ ID NO: 19 - DNA, 21 bp, synthetic construct
  source 1..21: mol_type = other DNA
agtgacgccaaggctgcggtg

SEQ ID NO: 20 - DNA, 17 bp, synthetic construct
  source 1..17: mol_type = other DNA
tgccgagcagcgcttct

SEQ ID NO: 21 - DNA, 22 bp, synthetic construct
  source 1..22: mol_type = other DNA
tgtactggaagaacttgcttac

SEQ ID NO: 22 - DNA, 25 bp, synthetic construct
  source 1..25: mol_type = other DNA
tgtagttgggaggtgaaataagttg

SEQ ID NO: 23 - DNA, 24 bp, synthetic construct
  source 1..24: mol_type = other DNA
cctgaggccagcatggtggtagtg

SEQ ID NO: 24 - DNA, 17 bp, synthetic construct
  source 1..17: mol_type = other DNA
tgacgccaaggctgcgg

SEQ ID NO: 25 - DNA, 25 bp, synthetic construct
  source 1..25: mol_type = other DNA
gtgtactggaagaacttgcttacct

SEQ ID NO: 26 - DNA, 456 bp, Homo sapiens
  source 1..456: mol_type = genomic DNA
gctggcactttctgttatgtttgtgttagtctcgtgtccttgggtgactctgggttgaaatctttaatgctcccccaagaggcttgctgtttgggctctctgaaagtgacgccaaggctgcggtgtccaccaactgccgagcagcgcttctccatggaggtaagcaagttcttccagtacaaactgaatggtcatgttaaaagcaagtcatttttacagccatacctatttttattgccctaccctacagagttcctttgggatcatcttttctcaacctgttctaaacacagtcatcagtgttttctcaccctcacttcaggctttactttctaaagtttgtagaatgaatatagttttcattacagaaataagtattgaatagttcttccagctatacatgtgtgctcctgccgacattttgataggcttctaatctcccttccttcttctccc

SEQ ID NO: 27 - DNA, 510 bp, Homo sapiens
  source 1..510: mol_type = genomic DNA
ccacagccctgcggcacccctcctgaagtaccacagatttagtctggaggccccctctctgttcagctgccctggggtccccttatcctcccttgctggctgtgtcccaagctaggcaggattcatggtggggcatgtagttgggaggtgaaatgaggtaattatgtaatcagccaaagtccatccctctttttcaggcagtataaaggcaaaccaccccagccgtcaccatctatcatcccactaccaccatgctggcctcagggatgcttctggtggccttgctggtctgcctgactgtaatggtcttgatgtctgtttggcagcagaggaagagcaaggggaagctgcctccgggacccaccccattgcccttcattggaaactacctgcagctgaacacagagcagatgtacaactccctcatgaaggtgtcccaaggcagggagatgggtggcacggggtgggggctgcctagttggctggggctttgtggcagggggttgacca

SEQ ID NO: 28 - DNA, 510 bp, Homo sapiens
  source 1..510: mol_type = genomic DNA
ccacagccctgcggcacccctcctgaagtaccacagatttagtctggaggccccctctctgttcagctgccctggggtccccttatcctcccttgctggctgtgtcccaagctaggcaggattcatggtggggcatgtagttgggaggtgaaatgaggtaattatgtaatcagccaaagtccatccctctttttcaggcagtagaaaggcaaaccaccccagccgtcaccatctatcatcccactaccaccatgctggcctcagggatgcttctggtggccttgctggtctgcctgactgtaatggtcttgatgtctgtttggcagcagaggaagagcaaggggaagctgcctccgggacccaccccattgcccttcattggaaactacctgcagctgaacacagagcagatgtacaactccctcatgaaggtgtcccaaggcagggagatgggtggcacggggtgggggctgcctagttggctggggctttgtggcagggggttgacca

SEQ ID NO: 29 - DNA, 767 bp, Homo sapiens
  source 1..767: mol_type = genomic DNA
ctccagatgcacagccacacttccatctcaccctaataaaacccagacctttggattcctctcccttggaatgcccaaatccacaactttggggtgcattctcactctcagaccccaaatccaaagcccaagtgctcccctatgcaaatattccaaactcttcagttctacagtttatcggttgccccctcctaaatccacagccctgcggcacccctcctgaagtaccacagatttagtctggaggccccctctctgttcagctgccctggggtccccttatcctcccttgctggctgtgtcccaagctaggtggcattcatggtggggcgtgtagttgggaggtgaaataaggtgattatgtaattagccaaagtccatccctctttttcaggcagtataaaggcaaaccaccccacccatcaccatctgtcatctcactaccaccatgctggcctcagggctgcttctggtggccttgctggcctgcctgactgtgatggtcttgatgtctgtctggcagcagaggaagagcagggggaagctgcctccgggacccaccccactgcccttcattggaaactacctccagctgaacacagagcacatatgtgactccatcatgaaggtgtcccaaggcaggaagatgggtggcacagggtgggggctgcctagttggctggggctttgtggcaggggattgaccagtgtggaccagagtcttaggaaagggagttttggagtttcagcatccgggtcctagccag